European Patent Application EP 4 331 678 A1, published March 6, 2024. Title: BCMA-TARGETING CHIMERIC ANTIGEN RECEPTOR AND USE THEREOF. Applicant: ORICELL THERAPEUTICS CO., LTD. The sequence listing filed with the application follows.

SEQUENCE LISTING (107 sequences)

SEQ ID NO: 1 - protein, 111 aa, Artificial Sequence
  VL
EIVLTQSPATLSLSPGERATLSCRASESVSVIGAHLIHWYQQKPGQAPRLLIYLGRNRAAGIPARFSGSGSGTDFTLTISSLEPEDAAIYYCLQSRIFPRTFGQGTKLEIK

SEQ ID NO: 2 - protein, 111 aa, Artificial Sequence
  VL
EIVLTQSPATLSLSPGERATLSCRASESVSVSGIHLLHWYQQKPGQAPRLLIYLGRNRAAGIPARFSGSGSGTDFTLTISSLEPEDAAIYYCLQSRRFPRHFGQGTKLEIK

SEQ ID NO: 3 - protein, 111 aa, Artificial Sequence
  VL
EIVLTQSPATLSLSPGERATLSCRASESVSVPGISFIHWYQQKPGQAPRLLIYLGRNRAAGIPARFSGSGSGTDFTLTISSLEPEDAAIYYCLQSRRFPRHFGQGTKLEIK

SEQ ID NO: 4 - protein, 111 aa, Artificial Sequence
  VL
EIVLTQSPATLSLSPGERATLSCRASESVSVPGISFIHWYQQKPGQAPRLLIYLGSNRPSGIPARFSGSGSGTDFTLTISSLEPEDAAIYYCLQSRRFPRHFGQGTKLEIK

SEQ ID NO: 5 - protein, 117 aa, Artificial Sequence
  VH
QVQLVQSGSELKKPGASVKVSCKASGYTFADYTINWVRQATGQGLEWMGWINTETREPAYAYDFRGRFVFSLDTSVSTAYLQISSLKAEDTAVYYCARDIRYVMDYWGQGTLVTVSS

SEQ ID NO: 6 - protein, 117 aa, Artificial Sequence
  VH
QVQLVQSGSELKKPGASVKVSCKASGYSFADYTINWVRQAPGQGLEWIGWINTETREPAYAYDFRSRFVFSLDTSASTAYLQISSLKAEDTAVYYCARDIRYVMDYWGQGTLVTVSS

SEQ ID NO: 7 - protein, 117 aa, Artificial Sequence
  VH
QVQLVQSGSEVKQPGASVKVSCKASGYSFADYTINWVRQAPGQGLEWMGWINTETREPTYAYDFRSRFVFSLDTSASTAYLELSSLRSEDTAVYYCARDIRYVMDYWGQGTLVTVSS

SEQ ID NO: 8 - protein, 117 aa, Artificial Sequence
  VH
QVQLVQSGAEVKKPGASVKVSCKASGYTFADYTINWVRQATGQGLEWMGWINTETREPTYAYDFRSRFTFTLNTSISTAYLELSSLRSEDTAVYYCARDIRYVMDYWGQGTLVTVSS

SEQ ID NO: 9 - protein, 117 aa, Artificial Sequence
  VH
QVQLVQSGAEVKKPGASVKVSCKASGYTFADYTINWVRQATGQGLEWMGWINTETREPAYAYDFRGRFTFTLNTSISTAYLELSSLRSEDTAVYYCARDIRYVMDYWGQGTLVTVSS

SEQ ID NO: 10 - protein, 15 aa, Artificial Sequence
  LCDR1
RASESVSVIGAHLIH

SEQ ID NO: 11 - protein, 15 aa, Artificial Sequence
  LCDR1
RASESVSVSGIHLLH

SEQ ID NO: 12 - protein, 15 aa, Artificial Sequence
  LCDR1
RASESVSVPGISFIH

SEQ ID NO: 13 - protein, 7 aa, Artificial Sequence
  LCDR2
LGRNRAA

SEQ ID NO: 14 - protein, 7 aa, Artificial Sequence
  LCDR2
LGSNRPS

SEQ ID NO: 15 - protein, 9 aa, Artificial Sequence
  LCDR3
LQSRIFPRT

SEQ ID NO: 16 - protein, 9 aa, Artificial Sequence
  LCDR3
LQSRRFPRH

SEQ ID NO: 17 - protein, 23 aa, Artificial Sequence
  L-FR1
EIVLTQSPATLSLSPGERATLSC

SEQ ID NO: 18 - protein, 15 aa, Artificial Sequence
  L-FR2
WYQQKPGQAPRLLIY

SEQ ID NO: 19 - protein, 32 aa, Artificial Sequence
  L-FR3
GIPARFSGSGSGTDFTLTISSLEPEDAAIYYC

SEQ ID NO: 20 - protein, 10 aa, Artificial Sequence
  L-FR4
FGQGTKLEIK

SEQ ID NO: 21 - protein, 5 aa, Artificial Sequence
  HCDR1
DYTIN

SEQ ID NO: 22 - protein, 17 aa, Artificial Sequence
  HCDR2
WINTETREPAYAYDFRG

SEQ ID NO: 23 - protein, 17 aa, Artificial Sequence
  HCDR2
WINTETREPAYAYDFRS

SEQ ID NO: 24 - protein, 17 aa, Artificial Sequence
  HCDR2
WINTETREPTYAYDFRS

SEQ ID NO: 25 - protein, 8 aa, Artificial Sequence
  HCDR3
DIRYVMDY

SEQ ID NO: 26 - protein, 30 aa, Artificial Sequence
  H-FR1
QVQLVQSGSELKKPGASVKVSCKASGYTFA

SEQ ID NO: 27 - protein, 30 aa, Artificial Sequence
  H-FR1
QVQLVQSGSELKKPGASVKVSCKASGYSFA

SEQ ID NO: 28 - protein, 30 aa, Artificial Sequence
  H-FR1
QVQLVQSGSEVKQPGASVKVSCKASGYSFA

SEQ ID NO: 29 - protein, 30 aa, Artificial Sequence
  H-FR1
QVQLVQSGAEVKKPGASVKVSCKASGYTFA

SEQ ID NO: 30 - protein, 14 aa, Artificial Sequence
  H-FR2
WVRQATGQGLEWMG

SEQ ID NO: 31 - protein, 14 aa, Artificial Sequence
  H-FR2
WVRQAPGQGLEWIG

SEQ ID NO: 32 - protein, 14 aa, Artificial Sequence
  H-FR2
WVRQAPGQGLEWMG

SEQ ID NO: 33 - protein, 32 aa, Artificial Sequence
  H-FR3
RFVFSLDTSVSTAYLQISSLKAEDTAVYYCAR

SEQ ID NO: 34 - protein, 32 aa, Artificial Sequence
  H-FR3
RFVFSLDTSASTAYLQISSLKAEDTAVYYCAR

SEQ ID NO: 35 - protein, 32 aa, Artificial Sequence
  H-FR3
RFVFSLDTSASTAYLELSSLRSEDTAVYYCAR

SEQ ID NO: 36 - protein, 32 aa, Artificial Sequence
  H-FR3
RFTFTLNTSISTAYLELSSLRSEDTAVYYCAR

SEQ ID NO: 37 - protein, 11 aa, Artificial Sequence
  H-FR4
WGQGTLVTVSS

SEQ ID NO: 38 - protein, 15 aa, Artificial Sequence
  LCDR1
  misc_feature (9)..(9): Xaa = Ile Pro or Ser
  misc_feature (11)..(11): Xaa = Ala or Ile
  misc_feature (12)..(12): Xaa = His or Ser
  misc_feature (13)..(13): Xaa = Phe or Leu
  misc_feature (14)..(14): Xaa = Ile or Leu
RASESVSVXGXXXXH

SEQ ID NO: 39 - protein, 7 aa, Artificial Sequence
  LCDR2
  misc_feature (3)..(3): Xaa = Arg or Ser
  misc_feature (6)..(6): Xaa = Ala or Pro
  misc_feature (7)..(7): Xaa = Ala or Ser
LGXNRXX

SEQ ID NO: 40 - protein, 9 aa, Artificial Sequence
  LCDR3
  misc_feature (5)..(5): Xaa = Ile or Arg
  misc_feature (9)..(9): Xaa = His or Thr
LQSRXFPRX

SEQ ID NO: 41 - protein, 17 aa, Artificial Sequence
  HCDR2
  misc_feature (10)..(10): Xaa = Ala or Thr
  misc_feature (17)..(17): Xaa = Gly or Ser
WINTETREPXYAYDFRX

SEQ ID NO: 42 - protein, 30 aa, Artificial Sequence
  H-FR1
  misc_feature (9)..(9): Xaa = Ala or Ser
  misc_feature (11)..(11): Xaa = Leu or Val
  misc_feature (13)..(13): Xaa = Lys or Gln
  misc_feature (28)..(28): Xaa = Ser or Thr
QVQLVQSGXEXKXPGASVKVSCKASGYXFA

SEQ ID NO: 43 - protein, 14 aa, Artificial Sequence
  H-FR2
  misc_feature (6)..(6): Xaa = Pro or Thr
  misc_feature (13)..(13): Xaa = Ile or Met
WVRQAXGQGLEWXG

SEQ ID NO: 44 - protein, 32 aa, Artificial Sequence
  H-FR3
  misc_feature (3)..(3): Xaa = Thr or Val
  misc_feature (5)..(5): Xaa = Ser or Thr
  misc_feature (7)..(7): Xaa = Asp or Asn
  misc_feature (10)..(10): Xaa = Ala Ile or Val
  misc_feature (16)..(16): Xaa = Glu or Gln
  misc_feature (17)..(17): Xaa = Ile or Leu
  misc_feature (21)..(21): Xaa = Lys or Arg
  misc_feature (22)..(22): Xaa = Ala or Ser
RFXFXLXTSXSTAYLXXSSLXXEDTAVYYCAR

SEQ ID NO: 45 - protein, 111 aa, Artificial Sequence
  VL
  misc_feature (32)..(32): Xaa = Ile Pro or Ser
  misc_feature (34)..(34): Xaa = Ala or Ile
  misc_feature (35)..(35): Xaa = His or Ser
  misc_feature (36)..(36): Xaa = Phe or Leu
  misc_feature (37)..(37): Xaa = Ile or Leu
  misc_feature (56)..(56): Xaa = Arg or Ser
  misc_feature (59)..(59): Xaa = Ala or Pro
  misc_feature (60)..(60): Xaa = Ala or Ser
  misc_feature (97)..(97): Xaa = Ile or Arg
  misc_feature (101)..(101): Xaa = His or Thr
EIVLTQSPATLSLSPGERATLSCRASESVSVXGXXXXHWYQQKPGQAPRLLIYLGXNRXXGIPARFSGSGSGTDFTLTISSLEPEDAAIYYCLQSRXFPRXFGQGTKLEIK

SEQ ID NO: 46 - protein, 117 aa, Artificial Sequence
  VH
  misc_feature (9)..(9): Xaa = Ala or Ser
  misc_feature (11)..(11): Xaa = Leu or Val
  misc_feature (13)..(13): Xaa = Lys or Gln
  misc_feature (28)..(28): Xaa = Ser or Thr
  misc_feature (41)..(41): Xaa = Pro or Thr
  misc_feature (48)..(48): Xaa = Ile or Met
  misc_feature (59)..(59): Xaa = Ala or Thr
  misc_feature (66)..(66): Xaa = Gly or Ser
  misc_feature (69)..(69): Xaa = Thr or Val
  misc_feature (71)..(71): Xaa = Ser or Thr
  misc_feature (73)..(73): Xaa = Asp or Asn
  misc_feature (76)..(76): Xaa = Ala Ile or Val
  misc_feature (82)..(82): Xaa = Glu or Gln
  misc_feature (83)..(83): Xaa = Ile or Leu
  misc_feature (87)..(87): Xaa = Lys or Arg
  misc_feature (88)..(88): Xaa = Ala or Ser
QVQLVQSGXEXKXPGASVKVSCKASGYXFADYTINWVRQAXGQGLEWXGWINTETREPXYAYDFRXRFXFXLXTSXSTAYLXXSSLXXEDTAVYYCARDIRYVMDYWGQGTLVTVSS

SEQ ID NO: 47 - protein, 111 aa, Artificial Sequence
  VL
DIVLTQSPASLAVSLGERATINCRASESVSVIGAHLIHWYQQKPGQPPKLLIYLASNLETGVPARFSGSGSGTDFTLTISSLQAEDAAIYYCLQSRIFPRTFGQGTKLEIK

SEQ ID NO: 48 - protein, 117 aa, Artificial Sequence
  VH
QVQLVQSGSELKKPGASVKVSCKASGYTFTDYSINWVRQAPGQGLEWMGWINTETREPAYAYDFRGRFVFSLDTSVSTAYLQISSLKAEDTAVYYCARDYSYAMDYWGQGTLVTVSS

SEQ ID NO: 49 - protein, 246 aa, Artificial Sequence
  hBCMA-01 scFv
EIVLTQSPATLSLSPGERATLSCRASESVSVIGAHLIHWYQQKPGQAPRLLIYLGRNRAAGIPARFSGSGSGTDFTLTISSLEPEDAAIYYCLQSRIFPRTFGQGTKLEIKGSTSGSGKPGSGEGSTKGQVQLVQSGSELKKPGASVKVSCKASGYTFADYTINWVRQATGQGLEWMGWINTETREPAYAYDFRGRFVFSLDTSVSTAYLQISSLKAEDTAVYYCARDIRYVMDYWGQGTLVTVSS

SEQ ID NO: 50 - protein, 246 aa, Artificial Sequence
  hBCMA-02 scFv
EIVLTQSPATLSLSPGERATLSCRASESVSVSGIHLLHWYQQKPGQAPRLLIYLGRNRAAGIPARFSGSGSGTDFTLTISSLEPEDAAIYYCLQSRRFPRHFGQGTKLEIKGSTSGSGKPGSGEGSTKGQVQLVQSGSELKKPGASVKVSCKASGYSFADYTINWVRQAPGQGLEWIGWINTETREPAYAYDFRSRFVFSLDTSASTAYLQISSLKAEDTAVYYCARDIRYVMDYWGQGTLVTVSS

SEQ ID NO: 51 - protein, 246 aa, Artificial Sequence
  hBCMA-15 scFv
EIVLTQSPATLSLSPGERATLSCRASESVSVSGIHLLHWYQQKPGQAPRLLIYLGRNRAAGIPARFSGSGSGTDFTLTISSLEPEDAAIYYCLQSRRFPRHFGQGTKLEIKGSTSGSGKPGSGEGSTKGQVQLVQSGSEVKQPGASVKVSCKASGYSFADYTINWVRQAPGQGLEWMGWINTETREPTYAYDFRSRFVFSLDTSASTAYLELSSLRSEDTAVYYCARDIRYVMDYWGQGTLVTVSS

SEQ ID NO: 52 - protein, 246 aa, Artificial Sequence
  hBCMA-17 scFv
EIVLTQSPATLSLSPGERATLSCRASESVSVSGIHLLHWYQQKPGQAPRLLIYLGRNRAAGIPARFSGSGSGTDFTLTISSLEPEDAAIYYCLQSRRFPRHFGQGTKLEIKGSTSGSGKPGSGEGSTKGQVQLVQSGAEVKKPGASVKVSCKASGYTFADYTINWVRQATGQGLEWMGWINTETREPTYAYDFRSRFTFTLNTSISTAYLELSSLRSEDTAVYYCARDIRYVMDYWGQGTLVTVSS

SEQ ID NO: 53 - protein, 246 aa, Artificial Sequence
  hBCMA-19 scFv
EIVLTQSPATLSLSPGERATLSCRASESVSVPGISFIHWYQQKPGQAPRLLIYLGRNRAAGIPARFSGSGSGTDFTLTISSLEPEDAAIYYCLQSRRFPRHFGQGTKLEIKGSTSGSGKPGSGEGSTKGQVQLVQSGAEVKKPGASVKVSCKASGYTFADYTINWVRQATGQGLEWMGWINTETREPAYAYDFRGRFTFTLNTSISTAYLELSSLRSEDTAVYYCARDIRYVMDYWGQGTLVTVSS

SEQ ID NO: 54 - protein, 246 aa, Artificial Sequence
  hBCMA-20 scFv
EIVLTQSPATLSLSPGERATLSCRASESVSVPGISFIHWYQQKPGQAPRLLIYLGRNRAAGIPARFSGSGSGTDFTLTISSLEPEDAAIYYCLQSRRFPRHFGQGTKLEIKGSTSGSGKPGSGEGSTKGQVQLVQSGAEVKKPGASVKVSCKASGYTFADYTINWVRQATGQGLEWMGWINTETREPTYAYDFRSRFTFTLNTSISTAYLELSSLRSEDTAVYYCARDIRYVMDYWGQGTLVTVSS

SEQ ID NO: 55 - protein, 246 aa, Artificial Sequence
  hBCMA-22 scFv
EIVLTQSPATLSLSPGERATLSCRASESVSVPGISFIHWYQQKPGQAPRLLIYLGSNRPSGIPARFSGSGSGTDFTLTISSLEPEDAAIYYCLQSRRFPRHFGQGTKLEIKGSTSGSGKPGSGEGSTKGQVQLVQSGAEVKKPGASVKVSCKASGYTFADYTINWVRQATGQGLEWMGWINTETREPAYAYDFRGRFTFTLNTSISTAYLELSSLRSEDTAVYYCARDIRYVMDYWGQGTLVTVSS

SEQ ID NO: 56 - protein, 246 aa, Artificial Sequence
  hBCMA-23 scFv
EIVLTQSPATLSLSPGERATLSCRASESVSVPGISFIHWYQQKPGQAPRLLIYLGSNRPSGIPARFSGSGSGTDFTLTISSLEPEDAAIYYCLQSRRFPRHFGQGTKLEIKGSTSGSGKPGSGEGSTKGQVQLVQSGAEVKKPGASVKVSCKASGYTFADYTINWVRQATGQGLEWMGWINTETREPTYAYDFRSRFTFTLNTSISTAYLELSSLRSEDTAVYYCARDIRYVMDYWGQGTLVTVSS

SEQ ID NO: 57 - protein, 231 aa, Homo sapiens
  human Fc
PKSCDKTHTCPPCPAPELLGGPSVFLFPPKPKDTLMISRTPEVTCVVVDVSHEDPEVKFNWYVDGVEVHNAKTKPREEQYNSTYRVVSVLTVLHQDWLNGKEYKCKVSNKALPAPIEKTISKAKGQPREPQVYTLPPSREEMTKNQVSLTCLVKGFYPSDIAVEWESNGQPENNYKTTPPVLDSDGSFFLYSKLTVDKSRWQQGNVFSCSVMHEALHNHYTQKSLSLSPGK

SEQ ID NO: 58 - protein, 18 aa, Artificial Sequence
  linker peptide
GSTSGSGKPGSGEGSTKG

SEQ ID NO: 59 - protein, 21 aa, Artificial Sequence
  signal peptide
MALPVTALLLPLALLLHAARP

SEQ ID NO: 60 - protein, 45 aa, Artificial Sequence
  CD8 hinge region
TTTPAPRPPTPAPTIASQPLSLRPEACRPAAGGAVHTRGLDFACD

SEQ ID NO: 61 - protein, 24 aa, Artificial Sequence
  CD8 transmembrane domain
IYIWAPLAGTCGVLLLSLVITLYC

SEQ ID NO: 62 - protein, 42 aa, Artificial Sequence
  CD137 costimulatory domain
KRGRKKLLYIFKQPFMRPVQTTQEEDGCSCRFPEEEEGGCEL

SEQ ID NO: 63 - protein, 112 aa, Artificial Sequence
  CD3zeta intracellular signaling domain
RVKFSRSADAPAYQQGQNQLYNELNLGRREEYDVLDKRRGRDPEMGGKPRRKNPQEGLYNELQKDKMAEAYSEIGMKGERRRGKGHDGLYQGLSTATKDTYDALHMQALPPR

SEQ ID NO: 64 - protein, 490 aa, Artificial Sequence
  hBCMA-01 CAR
MALPVTALLLPLALLLHAARPEIVLTQSPATLSLSPGERATLSCRASESVSVIGAHLIHWYQQKPGQAPRLLIYLGRNRAAGIPARFSGSGSGTDFTLTISSLEPEDAAIYYCLQSRIFPRTFGQGTKLEIKGSTSGSGKPGSGEGSTKGQVQLVQSGSELKKPGASVKVSCKASGYTFADYTINWVRQATGQGLEWMGWINTETREPAYAYDFRGRFVFSLDTSVSTAYLQISSLKAEDTAVYYCARDIRYVMDYWGQGTLVTVSSTTTPAPRPPTPAPTIASQPLSLRPEACRPAAGGAVHTRGLDFACDIYIWAPLAGTCGVLLLSLVITLYCKRGRKKLLYIFKQPFMRPVQTTQEEDGCSCRFPEEEEGGCELRVKFSRSADAPAYQQGQNQLYNELNLGRREEYDVLDKRRGRDPEMGGKPRRKNPQEGLYNELQKDKMAEAYSEIGMKGERRRGKGHDGLYQGLSTATKDTYDALHMQALPPR

SEQ ID NO: 65 - protein, 490 aa, Artificial Sequence
  hBCMA-02 CAR
MALPVTALLLPLALLLHAARPEIVLTQSPATLSLSPGERATLSCRASESVSVSGIHLLHWYQQKPGQAPRLLIYLGRNRAAGIPARFSGSGSGTDFTLTISSLEPEDAAIYYCLQSRRFPRHFGQGTKLEIKGSTSGSGKPGSGEGSTKGQVQLVQSGSELKKPGASVKVSCKASGYSFADYTINWVRQAPGQGLEWIGWINTETREPAYAYDFRSRFVFSLDTSASTAYLQISSLKAEDTAVYYCARDIRYVMDYWGQGTLVTVSSTTTPAPRPPTPAPTIASQPLSLRPEACRPAAGGAVHTRGLDFACDIYIWAPLAGTCGVLLLSLVITLYCKRGRKKLLYIFKQPFMRPVQTTQEEDGCSCRFPEEEEGGCELRVKFSRSADAPAYQQGQNQLYNELNLGRREEYDVLDKRRGRDPEMGGKPRRKNPQEGLYNELQKDKMAEAYSEIGMKGERRRGKGHDGLYQGLSTATKDTYDALHMQALPPR

SEQ ID NO: 66 - protein, 490 aa, Artificial Sequence
  hBCMA-15 CAR
MALPVTALLLPLALLLHAARPEIVLTQSPATLSLSPGERATLSCRASESVSVSGIHLLHWYQQKPGQAPRLLIYLGRNRAAGIPARFSGSGSGTDFTLTISSLEPEDAAIYYCLQSRRFPRHFGQGTKLEIKGSTSGSGKPGSGEGSTKGQVQLVQSGSEVKQPGASVKVSCKASGYSFADYTINWVRQAPGQGLEWMGWINTETREPTYAYDFRSRFVFSLDTSASTAYLELSSLRSEDTAVYYCARDIRYVMDYWGQGTLVTVSSTTTPAPRPPTPAPTIASQPLSLRPEACRPAAGGAVHTRGLDFACDIYIWAPLAGTCGVLLLSLVITLYCKRGRKKLLYIFKQPFMRPVQTTQEEDGCSCRFPEEEEGGCELRVKFSRSADAPAYQQGQNQLYNELNLGRREEYDVLDKRRGRDPEMGGKPRRKNPQEGLYNELQKDKMAEAYSEIGMKGERRRGKGHDGLYQGLSTATKDTYDALHMQALPPR

SEQ ID NO: 67 - protein, 490 aa, Artificial Sequence
  hBCMA-17 CAR
MALPVTALLLPLALLLHAARPEIVLTQSPATLSLSPGERATLSCRASESVSVSGIHLLHWYQQKPGQAPRLLIYLGRNRAAGIPARFSGSGSGTDFTLTISSLEPEDAAIYYCLQSRRFPRHFGQGTKLEIKGSTSGSGKPGSGEGSTKGQVQLVQSGAEVKKPGASVKVSCKASGYTFADYTINWVRQATGQGLEWMGWINTETREPTYAYDFRSRFTFTLNTSISTAYLELSSLRSEDTAVYYCARDIRYVMDYWGQGTLVTVSSTTTPAPRPPTPAPTIASQPLSLRPEACRPAAGGAVHTRGLDFACDIYIWAPLAGTCGVLLLSLVITLYCKRGRKKLLYIFKQPFMRPVQTTQEEDGCSCRFPEEEEGGCELRVKFSRSADAPAYQQGQNQLYNELNLGRREEYDVLDKRRGRDPEMGGKPRRKNPQEGLYNELQKDKMAEAYSEIGMKGERRRGKGHDGLYQGLSTATKDTYDALHMQALPPR

SEQ ID NO: 68 - protein, 490 aa, Artificial Sequence
  hBCMA-19 CAR
MALPVTALLLPLALLLHAARPEIVLTQSPATLSLSPGERATLSCRASESVSVPGISFIHWYQQKPGQAPRLLIYLGRNRAAGIPARFSGSGSGTDFTLTISSLEPEDAAIYYCLQSRRFPRHFGQGTKLEIKGSTSGSGKPGSGEGSTKGQVQLVQSGAEVKKPGASVKVSCKASGYTFADYTINWVRQATGQGLEWMGWINTETREPAYAYDFRGRFTFTLNTSISTAYLELSSLRSEDTAVYYCARDIRYVMDYWGQGTLVTVSSTTTPAPRPPTPAPTIASQPLSLRPEACRPAAGGAVHTRGLDFACDIYIWAPLAGTCGVLLLSLVITLYCKRGRKKLLYIFKQPFMRPVQTTQEEDGCSCRFPEEEEGGCELRVKFSRSADAPAYQQGQNQLYNELNLGRREEYDVLDKRRGRDPEMGGKPRRKNPQEGLYNELQKDKMAEAYSEIGMKGERRRGKGHDGLYQGLSTATKDTYDALHMQALPPR

SEQ ID NO: 69 - protein, 490 aa, Artificial Sequence
  hBCMA-20 CAR
MALPVTALLLPLALLLHAARPEIVLTQSPATLSLSPGERATLSCRASESVSVPGISFIHWYQQKPGQAPRLLIYLGRNRAAGIPARFSGSGSGTDFTLTISSLEPEDAAIYYCLQSRRFPRHFGQGTKLEIKGSTSGSGKPGSGEGSTKGQVQLVQSGAEVKKPGASVKVSCKASGYTFADYTINWVRQATGQGLEWMGWINTETREPTYAYDFRSRFTFTLNTSISTAYLELSSLRSEDTAVYYCARDIRYVMDYWGQGTLVTVSSTTTPAPRPPTPAPTIASQPLSLRPEACRPAAGGAVHTRGLDFACDIYIWAPLAGTCGVLLLSLVITLYCKRGRKKLLYIFKQPFMRPVQTTQEEDGCSCRFPEEEEGGCELRVKFSRSADAPAYQQGQNQLYNELNLGRREEYDVLDKRRGRDPEMGGKPRRKNPQEGLYNELQKDKMAEAYSEIGMKGERRRGKGHDGLYQGLSTATKDTYDALHMQALPPR

SEQ ID NO: 70 - protein, 490 aa, Artificial Sequence
  hBCMA-22 CAR
MALPVTALLLPLALLLHAARPEIVLTQSPATLSLSPGERATLSCRASESVSVPGISFIHWYQQKPGQAPRLLIYLGSNRPSGIPARFSGSGSGTDFTLTISSLEPEDAAIYYCLQSRRFPRHFGQGTKLEIKGSTSGSGKPGSGEGSTKGQVQLVQSGAEVKKPGASVKVSCKASGYTFADYTINWVRQATGQGLEWMGWINTETREPAYAYDFRGRFTFTLNTSISTAYLELSSLRSEDTAVYYCARDIRYVMDYWGQGTLVTVSSTTTPAPRPPTPAPTIASQPLSLRPEACRPAAGGAVHTRGLDFACDIYIWAPLAGTCGVLLLSLVITLYCKRGRKKLLYIFKQPFMRPVQTTQEEDGCSCRFPEEEEGGCELRVKFSRSADAPAYQQGQNQLYNELNLGRREEYDVLDKRRGRDPEMGGKPRRKNPQEGLYNELQKDKMAEAYSEIGMKGERRRGKGHDGLYQGLSTATKDTYDALHMQALPPR

SEQ ID NO: 71 - protein, 490 aa, Artificial Sequence
  hBCMA-23 CAR
MALPVTALLLPLALLLHAARPEIVLTQSPATLSLSPGERATLSCRASESVSVPGISFIHWYQQKPGQAPRLLIYLGSNRPSGIPARFSGSGSGTDFTLTISSLEPEDAAIYYCLQSRRFPRHFGQGTKLEIKGSTSGSGKPGSGEGSTKGQVQLVQSGAEVKKPGASVKVSCKASGYTFADYTINWVRQATGQGLEWMGWINTETREPTYAYDFRSRFTFTLNTSISTAYLELSSLRSEDTAVYYCARDIRYVMDYWGQGTLVTVSSTTTPAPRPPTPAPTIASQPLSLRPEACRPAAGGAVHTRGLDFACDIYIWAPLAGTCGVLLLSLVITLYCKRGRKKLLYIFKQPFMRPVQTTQEEDGCSCRFPEEEEGGCELRVKFSRSADAPAYQQGQNQLYNELNLGRREEYDVLDKRRGRDPEMGGKPRRKNPQEGLYNELQKDKMAEAYSEIGMKGERRRGKGHDGLYQGLSTATKDTYDALHMQALPPR

SEQ ID NO: 72 - protein, 490 aa, Artificial Sequence
  hBCMA-10 CAR
MALPVTALLLPLALLLHAARPDIVLTQSPASLAVSLGERATINCRASESVSVIGAHLIHWYQQKPGQPPKLLIYLASNLETGVPARFSGSGSGTDFTLTISSLQAEDAAIYYCLQSRIFPRTFGQGTKLEIKGSTSGSGKPGSGEGSTKGQVQLVQSGSELKKPGASVKVSCKASGYTFTDYSINWVRQAPGQGLEWMGWINTETREPAYAYDFRGRFVFSLDTSVSTAYLQISSLKAEDTAVYYCARDYSYAMDYWGQGTLVTVSSTTTPAPRPPTPAPTIASQPLSLRPEACRPAAGGAVHTRGLDFACDIYIWAPLAGTCGVLLLSLVITLYCKRGRKKLLYIFKQPFMRPVQTTQEEDGCSCRFPEEEEGGCELRVKFSRSADAPAYQQGQNQLYNELNLGRREEYDVLDKRRGRDPEMGGKPRRKNPQEGLYNELQKDKMAEAYSEIGMKGERRRGKGHDGLYQGLSTATKDTYDALHMQALPPR

SEQ ID NO: 73 - protein, 1098 aa, Artificial Sequence
  huBCMA-10-L6-Li CAR
MALPVTALLLPLALLLHAARPDIVLTQSPASLAVSLGERATINCRASESVSVIGAHLIHWYQQKPGQPPKLLIYLASNLETGVPARFSGSGSGTDFTLTISSLQAEDAAIYYCLQSRIFPRTFGQGTKLEIKGSTSGSGKPGSGEGSTKGQVQLVQSGSELKKPGASVKVSCKASGYTFTDYSINWVRQAPGQGLEWMGWINTETREPAYAYDFRGRFVFSLDTSVSTAYLQISSLKAEDTAVYYCARDYSYAMDYWGQGTLVTVSSTTTPAPRPPTPAPTIASQPLSLRPEACRPAAGGAVHTRGLDFACDIYIWAPLAGTCGVLLLSLVITLYCKRGRKKLLYIFKQPFMRPVQTTQEEDGCSCRFPEEEEGGCELRVKFSRSADAPAYQQGQNQLYNELNLGRREEYDVLDKRRGRDPEMGGKPRRKNPQEGLYNELQKDKMAEAYSEIGMKGERRRGKGHDGLYQGLSTATKDTYDALHMQALPPREGRGSLLTCGDVEENPGPMGAVLRSLLACSFCVLLRAEQKLISEEDLEPPTCSPQQFTCFTGEIDCIPVAWRCDGFTECEDHSDELNCPVCSESQFQCASGQCIDGALRCNGDANCQDKSDEKNCEVLCLIDQFRCANGQCIGKHKKCDHNVDCSDKSDELDCYPTEEPAPQATNTVGSVIGVIVTIFVSGTVYFICQRMLCPRMKGDGETMTNDYVVHGPASVPLGYVPHPSSLSGSLPGMSRGKSMISSLSIMGGSSGPPYDRAHVTGASSSSSSSTKGTYFPAILNPPPSPATERSHYTMEFGYSSNSPSTHRSYSYRPYSYRHFAPPTTPCSTDVCDSDYAPSRRMTSVATAKGYTSDLNYDSEPVPPPPTPRSQYLSAEENYESCPPSPYTERSYSHHLYPPPPSPCTDSSATNFSLLKQAGDVEENPGPMHWGTLCGFLWLWPYLFYVQAVPIQKVQDDTKTLIKTIVTRINDISHTQSVSSKQKVTGLDFIPGLHPILTLSKMDQTLAVYQQILTSMPSRNVIQISNDLENLRDLLHVLAFSKSCHLPWASGLETLDSLGGVLEASGYSTEVVALSRLQGSLQDMLWQLDLSPGCHHHHHH

SEQ ID NO: 74 - protein, 1098 aa, Artificial Sequence
  hBCMA-22-L6-Li CAR
MALPVTALLLPLALLLHAARPEIVLTQSPATLSLSPGERATLSCRASESVSVPGISFIHWYQQKPGQAPRLLIYLGSNRPSGIPARFSGSGSGTDFTLTISSLEPEDAAIYYCLQSRRFPRHFGQGTKLEIKGSTSGSGKPGSGEGSTKGQVQLVQSGAEVKKPGASVKVSCKASGYTFADYTINWVRQATGQGLEWMGWINTETREPAYAYDFRGRFTFTLNTSISTAYLELSSLRSEDTAVYYCARDIRYVMDYWGQGTLVTVSSTTTPAPRPPTPAPTIASQPLSLRPEACRPAAGGAVHTRGLDFACDIYIWAPLAGTCGVLLLSLVITLYCKRGRKKLLYIFKQPFMRPVQTTQEEDGCSCRFPEEEEGGCELRVKFSRSADAPAYQQGQNQLYNELNLGRREEYDVLDKRRGRDPEMGGKPRRKNPQEGLYNELQKDKMAEAYSEIGMKGERRRGKGHDGLYQGLSTATKDTYDALHMQALPPREGRGSLLTCGDVEENPGPMGAVLRSLLACSFCVLLRAEQKLISEEDLEPPTCSPQQFTCFTGEIDCIPVAWRCDGFTECEDHSDELNCPVCSESQFQCASGQCIDGALRCNGDANCQDKSDEKNCEVLCLIDQFRCANGQCIGKHKKCDHNVDCSDKSDELDCYPTEEPAPQATNTVGSVIGVIVTIFVSGTVYFICQRMLCPRMKGDGETMTNDYVVHGPASVPLGYVPHPSSLSGSLPGMSRGKSMISSLSIMGGSSGPPYDRAHVTGASSSSSSSTKGTYFPAILNPPPSPATERSHYTMEFGYSSNSPSTHRSYSYRPYSYRHFAPPTTPCSTDVCDSDYAPSRRMTSVATAKGYTSDLNYDSEPVPPPPTPRSQYLSAEENYESCPPSPYTERSYSHHLYPPPPSPCTDSSATNFSLLKQAGDVEENPGPMHWGTLCGFLWLWPYLFYVQAVPIQKVQDDTKTLIKTIVTRINDISHTQSVSSKQKVTGLDFIPGLHPILTLSKMDQTLAVYQQILTSMPSRNVIQISNDLENLRDLLHVLAFSKSCHLPWASGLETLDSLGGVLEASGYSTEVVALSRLQGSLQDMLWQLDLSPGCHHHHHH

SEQ ID NO: 75 - DNA, 333 bp, Artificial Sequence
  VL
gaaatcgttctgacccagagtccagcgacgctgagtctgagtccgggtgaacgcgcgacgctgagttgccgtgccagcgaaagcgttagcgtgattggcgcccatctgatccactggtaccagcagaaaccgggccaagccccacgtctgctgatctatctgggacgcaatcgggcggccggcattccagcccgctttagcggcagcggtagcggtaccgattttacgctgaccatcagcagtctggagccagaagatgccgccatctactactgtctgcagagccgcatcttcccacgcaccttcggccaaggcaccaaactggaaatcaag

SEQ ID NO: 76 - DNA, 333 bp, Artificial Sequence
  VL
gaaatcgttctgacccagagtccagcgacgctgagtctgagtccgggtgaacgcgcgacgctgagttgccgtgccagcgaaagcgttagcgtgagtggcattcacttactccactggtaccagcagaaaccgggccaagccccacgtctgctgatctatctgggacgcaatcgggcggccggcattccagcccgctttagcggcagcggtagcggtaccgattttacgctgaccatcagcagtctggagccagaagatgccgccatctactactgtttacagagcagaaggtttcctcgacacttcggccaaggtaccaaactggaaatcaag

SEQ ID NO: 77 - DNA, 333 bp, Artificial Sequence
  VL
gaaatcgttctgacccagagtccagcgacgctgagtctgagtccgggtgaacgcgcgacgctgagttgccgtgccagcgaaagcgttagcgtgcctggcatatctttcatccactggtaccagcagaaaccgggccaagccccacgtctgctgatctatctgggacgcaatcgggcggccggcattccagcccgctttagcggcagcggtagcggtaccgattttacgctgaccatcagcagtctggagccagaagatgccgccatctactactgtttacagagcagaaggtttcctcgacacttcggccaaggtaccaaactggaaatcaag

SEQ ID NO: 78 - DNA, 333 bp, Artificial Sequence
  VL
gaaatcgttctgacccagagtccagcgacgctgagtctgagtccgggtgaacgcgcgacgctgagttgccgtgccagcgaaagcgttagcgtgcctggcatatctttcatccactggtaccagcagaaaccgggccaagccccacgtctgctgatctatctgggcagcaatcgaccatccggcattccagcccgctttagcggcagcggtagcggtaccgattttacgctgaccatcagcagtctggagccagaagatgccgccatctactactgtttacagagcagaaggtttcctcgacacttcggccaaggcaccaaactggaaatcaag

SEQ ID NO: 79 - DNA, 333 bp, Artificial Sequence
  VL
gacatcgtgctgacccagagccccgcttctttagctgtgtctttaggagagagggccaccatcaattgtcgtgcctccgagtccgtgtccgtgattggcgcccatttaatccactggtaccagcagaaacccggccagccccccaagctgctgatctatttagccagcaatctggagaccggcgtgcccgccagatttagcggaagcggctccggcaccgattttactttaaccatttcctctttacaagctgaggacgccgccatctactactgtttacagagcagaatctttcctcgtaccttcggccaaggtaccaagctggaaatcaag

SEQ ID NO: 80 - DNA, 351 bp, Artificial Sequence
  VH
caagttcagctcgtgcagagcggctccgagctgaagaagcccggcgcttccgtgaaggtgagctgcaaggccagcggatacaccttcgccgattacaccatcaactgggttcgtcaagctaccggtcaaggtctggagtggatgggctggatcaacaccgaaaccagagagcccgcctatgcctacgacttcagaggtcgtttcgtgttctctttagacacaagcgtgagcaccgcctatttacagatcagctctttaaaggccgaggataccgccgtgtactactgcgctcgtgacatcagatacgtgatggactactggggccaaggtacactggtgaccgtgtccagc

SEQ ID NO: 81 - DNA, 351 bp, Artificial Sequence
  VH
caagttcagctcgtgcagagcggctccgagctgaagaagcccggcgcttccgtgaaggtgagctgcaaggccagcggatacagcttcgccgattacaccatcaactgggttcgtcaagctcccggtcaaggtctggagtggataggctggatcaacaccgaaaccagagagcccgcctatgcctacgacttcagaagtcgtttcgtgttctctttagacacaagcgcgagcaccgcctatttacagatcagctctttaaaggccgaggataccgccgtgtactactgcgctcgtgacatcagatacgtgatggactactggggccaaggtacactggtgaccgtgtccagc

SEQ ID NO: 82 - DNA, 351 bp, Artificial Sequence
  VH
caagttcagctcgtgcagagcggctccgaggtgaagcagcccggcgcttccgtgaaggtgagctgcaaggccagcggatacagcttcgccgattacaccatcaactgggttcgtcaagctcccggtcaaggtctggagtggatgggctggatcaacaccgaaaccagagagcccacctatgcctacgacttcagaagtcgtttcgtgttctctttagacacaagcgcgagcaccgcctatttagagctcagctctttaaggtccgaggataccgccgtgtactactgcgctcgtgacatcagatacgtgatggactactggggccaaggtacactggtgaccgtgtccagc

SEQ ID NO: 83 - DNA, 351 bp, Artificial Sequence
  VH
caagttcagctcgtgcagagcggcgccgaggtgaagaagcccggcgcttccgtgaaggtgagctgcaaggccagcggatacaccttcgccgattacaccatcaactgggttcgtcaagctaccggtcaaggtctggagtggatgggctggatcaacaccgaaaccagagagcccacctatgcctacgacttcagaagtcgtttcacgttcactttaaacacaagcatcagcaccgcctatttagagctcagctctttaaggtccgaggataccgccgtgtactactgcgctcgtgacatcagatacgtgatggactactggggccaaggtacactggtgaccgtgtccagc

SEQ ID NO: 84 - DNA, 351 bp, Artificial Sequence
  VH
caagttcagctcgtgcagagcggcgccgaggtgaagaagcccggcgcttccgtgaaggtgagctgcaaggccagcggatacaccttcgccgattacaccatcaactgggttcgtcaagctaccggtcaaggtctggagtggatgggctggatcaacaccgaaaccagagagcccgcctatgcctacgacttcagaggtcgtttcacgttcactttaaacacaagcatcagcaccgcctatttagagctcagctctttaaggtccgaggataccgccgtgtactactgcgctcgtgacatcagatacgtgatggactactggggccaaggtacactggtgaccgtgtccagc

SEQ ID NO: 85 - DNA, 351 bp, Artificial Sequence
  VH
caagttcagctcgtgcagagcggctccgagctgaagaagcccggcgcttccgtgaaggtgagctgcaaggccagcggatacaccttcaccgactactccatcaactgggttcgtcaagctcccggtcaaggtctggagtggatgggctggatcaacaccgaaaccagagagcccgcctatgcctacgacttcagaggtcgtttcgtgttctctttagacacaagcgtgagcaccgcctatttacagatcagctctttaaaggccgaggataccgccgtgtactactgcgctcgtgactacagctacgccatggactactggggccaaggtacactggtgaccgtgtccagc

SEQ ID NO: 86 - DNA, 54 bp, Artificial Sequence
  nucleotides of linker peptides
ggatccaccagcggctccggaaagcccggttccggagagggcagcacaaagggc

SEQ ID NO: 87 - DNA, 51 bp, Artificial Sequence
  forward primer
cctctggctctgctgctgcacgccgcaagacctgaaatcgttctgacccag

SEQ ID NO: 88 - DNA, 58 bp, Artificial Sequence
  reverse primer
tgggcgccggtgttggtggtcgcggcgctggcgtcgtggtgctggacacggtcaccag

SEQ ID NO: 89 - DNA, 735 bp, Artificial Sequence
  signal peptide-CD8 hinge region-CD8 transmembrane domain-CD137 costimulatory domain-CD3zeta intracellular signaling domain
atggctctgcctgtgaccgctctgctgctgcctctggctctgctgctgcacgccgcaagacctaccacgacgccagcgccgcgaccaccaacaccggcgcccaccatcgcgtcgcagcccctgtccctgcgcccagaggcgtgccggccagcggcggggggcgcagtgcacacgagggggctggacttcgcctgtgatatctacatctgggcgcccttggccgggacttgtggggtccttctcctgtcactggttatcaccctttactgcaaacggggcagaaagaaactcctgtatatattcaaacaaccatttatgagaccagtacaaactactcaagaggaagatggctgtagctgccgatttccagaagaagaagaaggaggatgtgaactgagagtgaagttcagcaggagcgcagacgcccccgcgtaccagcagggccagaaccagctctataacgagctcaatctaggacgaagagaggagtacgatgttttggacaagagacgtggccgggaccctgagatggggggaaagccgagaaggaagaaccctcaggaaggcctgtacaatgaactgcagaaagataagatggcggaggcctacagtgagattgggatgaaaggcgagcgccggaggggcaaggggcacgatggcctttaccagggtctcagtacagccaccaaggacacctacgacgcccttcacatgcaggccctgccccctcgctaa

SEQ ID NO: 90 - DNA, 63 bp, Artificial Sequence
  signal peptide
atggctctgcctgtgaccgctctgctgctgcctctggctctgctgctgcacgccgcaagacct

SEQ ID NO: 91 - DNA, 135 bp, Artificial Sequence
  CD8 hinge region
accacgacgccagcgccgcgaccaccaacaccggcgcccaccatcgcgtcgcagcccctgtccctgcgcccagaggcgtgccggccagcggcggggggcgcagtgcacacgagggggctggacttcgcctgtgat

SEQ ID NO: 92 - DNA, 72 bp, Artificial Sequence
  CD8 transmembrane domain
atctacatctgggcgcccttggccgggacttgtggggtccttctcctgtcactggttatcaccctttactgc

SEQ ID NO: 93 - DNA, 126 bp, Artificial Sequence
  CD137 costimulatory domain
aaacggggcagaaagaaactcctgtatatattcaaacaaccatttatgagaccagtacaaactactcaagaggaagatggctgtagctgccgatttccagaagaagaagaaggaggatgtgaactg

SEQ ID NO: 94 - DNA, 339 bp, Artificial Sequence
  CD3zeta intracellular signaling domain
agagtgaagttcagcaggagcgcagacgcccccgcgtaccagcagggccagaaccagctctataacgagctcaatctaggacgaagagaggagtacgatgttttggacaagagacgtggccgggaccctgagatggggggaaagccgagaaggaagaaccctcaggaaggcctgtacaatgaactgcagaaagataagatggcggaggcctacagtgagattgggatgaaaggcgagcgccggaggggcaaggggcacgatggcctttaccagggtctcagtacagccaccaaggacacctacgacgcccttcacatgcaggccctgccccctcgctaa

SEQ ID NO: 95 - DNA, 1473 bp, Artificial Sequence
  hBCMA-01 CAR
atggctctgcctgtgaccgctctgctgctgcctctggctctgctgctgcacgccgcaagacctgaaatcgttctgacccagagtccagcgacgctgagtctgagtccgggtgaacgcgcgacgctgagttgccgtgccagcgaaagcgttagcgtgattggcgcccatctgatccactggtaccagcagaaaccgggccaagccccacgtctgctgatctatctgggacgcaatcgggcggccggcattccagcccgctttagcggcagcggtagcggtaccgattttacgctgaccatcagcagtctggagccagaagatgccgccatctactactgtctgcagagccgcatcttcccacgcaccttcggccaaggcaccaaactggaaatcaagggatccaccagcggctccggaaagcccggttccggagagggcagcacaaagggccaagttcagctcgtgcagagcggctccgagctgaagaagcccggcgcttccgtgaaggtgagctgcaaggccagcggatacaccttcgccgattacaccatcaactgggttcgtcaagctaccggtcaaggtctggagtggatgggctggatcaacaccgaaaccagagagcccgcctatgcctacgacttcagaggtcgtttcgtgttctctttagacacaagcgtgagcaccgcctatttacagatcagctctttaaaggccgaggataccgccgtgtactactgcgctcgtgacatcagatacgtgatggactactggggccaaggtacactggtgaccgtgtccagcaccacgacgccagcgccgcgaccaccaacaccggcgcccaccatcgcgtcgcagcccctgtccctgcgcccagaggcgtgccggccagcggcggggggcgcagtgcacacgagggggctggacttcgcctgtgatatctacatctgggcgcccttggccgggacttgtggggtccttctcctgtcactggttatcaccctttactgcaaacggggcagaaagaaactcctgtatatattcaaacaaccatttatgagaccagtacaaactactcaagaggaagatggctgtagctgccgatttccagaagaagaagaaggaggatgtgaactgagagtgaagttcagcaggagcgcagacgcccccgcgtaccagcagggccagaaccagctctataacgagctcaatctaggacgaagagaggagtacgatgttttggacaagagacgtggccgggaccctgagatggggggaaagccgagaaggaagaaccctcaggaaggcctgtacaatgaactgcagaaagataagatggcggaggcctacagtgagattgggatgaaaggcgagcgccggaggggcaaggggcacgatggcctttaccagggtctcagtacagccaccaaggacacctacgacgcccttcacatgcaggccctgccccctcgctaa

SEQ ID NO: 96 - DNA, 1473 bp, Artificial Sequence
  hBCMA-02 CAR
atggctctgcctgtgaccgctctgctgctgcctctggctctgctgctgcacgccgcaagacctgaaatcgttctgacccagagtccagcgacgctgagtctgagtccgggtgaacgcgcgacgctgagttgccgtgccagcgaaagcgttagcgtgagtggcattcacttactccactggtaccagcagaaaccgggccaagccccacgtctgctgatctatctgggacgcaatcgggcggccggcattccagcccgctttagcggcagcggtagcggtaccgattttacgctgaccatcagcagtctggagccagaagatgccgccatctactactgtttacagagcagaaggtttcctcgacacttcggccaaggtaccaaactggaaatcaagggatccaccagcggctccggaaagcccggttccggagagggcagcacaaagggccaagttcagctcgtgcagagcggctccgagctgaagaagcccggcgcttccgtgaaggtgagctgcaaggccagcggatacagcttcgccgattacaccatcaactgggttcgtcaagctcccggtcaaggtctggagtggataggctggatcaacaccgaaaccagagagcccgcctatgcctacgacttcagaagtcgtttcgtgttctctttagacacaagcgcgagcaccgcctatttacagatcagctctttaaaggccgaggataccgccgtgtactactgcgctcgtgacatcagatacgtgatggactactggggccaaggtacactggtgaccgtgtccagcaccacgacgccagcgccgcgaccaccaacaccggcgcccaccatcgcgtcgcagcccctgtccctgcgcccagaggcgtgccggccagcggcggggggcgcagtgcacacgagggggctggacttcgcctgtgatatctacatctgggcgcccttggccgggacttgtggggtccttctcctgtcactggttatcaccctttactgcaaacggggcagaaagaaactcctgtatatattcaaacaaccatttatgagaccagtacaaactactcaagaggaagatggctgtagctgccgatttccagaagaagaagaaggaggatgtgaactgagagtgaagttcagcaggagcgcagacgcccccgcgtaccagcagggccagaaccagctctataacgagctcaatctaggacgaagagaggagtacgatgttttggacaagagacgtggccgggaccctgagatggggggaaagccgagaaggaagaaccctcaggaaggcctgtacaatgaactgcagaaagataagatggcggaggcctacagtgagattgggatgaaaggcgagcgccggaggggcaaggggcacgatggcctttaccagggtctcagtacagccaccaaggacacctacgacgcccttcacatgcaggccctgccccctcgctaa

SEQ ID NO: 97 - DNA, 1473 bp, Artificial Sequence
  hBCMA-15 CAR
atggctctgcctgtgaccgctctgctgctgcctctggctctgctgctgcacgccgcaagacctgaaatcgttctgacccagagtccagcgacgctgagtctgagtccgggtgaacgcgcgacgctgagttgccgtgccagcgaaagcgttagcgtgagtggcattcacttactccactggtaccagcagaaaccgggccaagccccacgtctgctgatctatctgggacgcaatcgggcggccggcattccagcccgctttagcggcagcggtagcggtaccgattttacgctgaccatcagcagtctggagccagaagatgccgccatctactactgtttacagagcagaaggtttcctcgacacttcggccaaggtaccaaactggaaatcaagggatccaccagcggctccggaaagcccggttccggagagggcagcacaaagggccaagttcagctcgtgcagagcggctccgaggtgaagcagcccggcgcttccgtgaaggtgagctgcaaggccagcggatacagcttcgccgattacaccatcaactgggttcgtcaagctcccggtcaaggtctggagtggatgggctggatcaacaccgaaaccagagagcccacctatgcctacgacttcagaagtcgtttcgtgttctctttagacacaagcgcgagcaccgcctatttagagctcagctctttaaggtccgaggataccgccgtgtactactgcgctcgtgacatcagatacgtgatggactactggggccaaggtacactggtgaccgtgtccagcaccacgacgccagcgccgcgaccaccaacaccggcgcccaccatcgcgtcgcagcccctgtccctgcgcccagaggcgtgccggccagcggcggggggcgcagtgcacacgagggggctggacttcgcctgtgatatctacatctgggcgcccttggccgggacttgtggggtccttctcctgtcactggttatcaccctttactgcaaacggggcagaaagaaactcctgtatatattcaaacaaccatttatgagaccagtacaaactactcaagaggaagatggctgtagctgccgatttccagaagaagaagaaggaggatgtgaactgagagtgaagttcagcaggagcgcagacgcccccgcgtaccagcagggccagaaccagctctataacgagctcaatctaggacgaagagaggagtacgatgttttggacaagagacgtggccgggaccctgagatggggggaaagccgagaaggaagaaccctcaggaaggcctgtacaatgaactgcagaaagataagatggcggaggcctacagtgagattgggatgaaaggcgagcgccggaggggcaaggggcacgatggcctttaccagggtctcagtacagccaccaaggacacctacgacgcccttcacatgcaggccctgccccctcgctaa

SEQ ID NO: 98 - DNA, 1473 bp, Artificial Sequence
  hBCMA-17 CAR
atggctctgcctgtgaccgctctgctgctgcctctggctctgctgctgcacgccgcaagacctgaaatcgttctgacccagagtccagcgacgctgagtctgagtccgggtgaacgcgcgacgctgagttgccgtgccagcgaaagcgttagcgtgagtggcattcacttactccactggtaccagcagaaaccgggccaagccccacgtctgctgatctatctgggacgcaatcgggcggccggcattccagcccgctttagcggcagcggtagcggtaccgattttacgctgaccatcagcagtctggagccagaagatgccgccatctactactgtttacagagcagaaggtttcctcgacacttcggccaaggtaccaaactggaaatcaagggatccaccagcggctccggaaagcccggttccggagagggcagcacaaagggccaagttcagctcgtgcagagcggcgccgaggtgaagaagcccggcgcttccgtgaaggtgagctgcaaggccagcggatacaccttcgccgattacaccatcaactgggttcgtcaagctaccggtcaaggtctggagtggatgggctggatcaacaccgaaaccagagagcccacctatgcctacgacttcagaagtcgtttcacgttcactttaaacacaagcatcagcaccgcctatttagagctcagctctttaaggtccgaggataccgccgtgtactactgcgctcgtgacatcagatacgtgatggactactggggccaaggtacactggtgaccgtgtccagcaccacgacgccagcgccgcgaccaccaacaccggcgcccaccatcgcgtcgcagcccctgtccctgcgcccagaggcgtgccggccagcggcggggggcgcagtgcacacgagggggctggacttcgcctgtgatatctacatctgggcgcccttggccgggacttgtggggtccttctcctgtcactggttatcaccctttactgcaaacggggcagaaagaaactcctgtatatattcaaacaaccatttatgagaccagtacaaactactcaagaggaagatggctgtagctgccgatttccagaagaagaagaaggaggatgtgaactgagagtgaagttcagcaggagcgcagacgcccccgcgtaccagcagggccagaaccagctctataacgagctcaatctaggacgaagagaggagtacgatgttttggacaagagacgtggccgggaccctgagatggggggaaagccgagaaggaagaaccctcaggaaggcctgtacaatgaactgcagaaagataagatggcggaggcctacagtgagattgggatgaaaggcgagcgccggaggggcaaggggcacgatggcctttaccagggtctcagtacagccaccaaggacacctacgacgcccttcacatgcaggccctgccccctcgctaa

SEQ ID NO: 99 - DNA, 1473 bp, Artificial Sequence
  hBCMA-19 CAR
atggctctgcctgtgaccgctctgctgctgcctctggctctgctgctgcacgccgcaagacctgaaatcgttctgacccagagtccagcgacgctgagtctgagtccgggtgaacgcgcgacgctgagttgccgtgccagcgaaagcgttagcgtgcctggcatatctttcatccactggtaccagcagaaaccgggccaagccccacgtctgctgatctatctgggacgcaatcgggcggccggcattccagcccgctttagcggcagcggtagcggtaccgattttacgctgaccatcagcagtctggagccagaagatgccgccatctactactgtttacagagcagaaggtttcctcgacacttcggccaaggtaccaaactggaaatcaagggatccaccagcggctccggaaagcccggttccggagagggcagcacaaagggccaagttcagctcgtgcagagcggcgccgaggtgaagaagcccggcgcttccgtgaaggtgagctgcaaggccagcggatacaccttcgccgattacaccatcaactgggttcgtcaagctaccggtcaaggtctggagtggatgggctggatcaacaccgaaaccagagagcccgcctatgcctacgacttcagaggtcgtttcacgttcactttaaacacaagcatcagcaccgcctatttagagctcagctctttaaggtccgaggataccgccgtgtactactgcgctcgtgacatcagatacgtgatggactactggggccaaggtacactggtgaccgtgtccagcaccacgacgccagcgccgcgaccaccaacaccggcgcccaccatcgcgtcgcagcccctgtccctgcgcccagaggcgtgccggccagcggcggggggcgcagtgcacacgagggggctggacttcgcctgtgatatctacatctgggcgcccttggccgggacttgtggggtccttctcctgtcactggttatcaccctttactgcaaacggggcagaaagaaactcctgtatatattcaaacaaccatttatgagaccagtacaaactactcaagaggaagatggctgtagctgccgatttccagaagaagaagaaggaggatgtgaactgagagtgaagttcagcaggagcgcagacgcccccgcgtaccagcagggccagaaccagctctataacgagctcaatctaggacgaagagaggagtacgatgttttggacaagagacgtggccgggaccctgagatggggggaaagccgagaaggaagaaccctcaggaaggcctgtacaatgaactgcagaaagataagatggcggaggcctacagtgagattgggatgaaaggcgagcgccggaggggcaaggggcacgatggcctttaccagggtctcagtacagccaccaaggacacctacgacgcccttcacatgcaggccctgccccctcgctaa

SEQ ID NO: 100 - DNA, 1473 bp, Artificial Sequence
  hBCMA-20 CAR
atggctctgcctgtgaccgctctgctgctgcctctggctctgctgctgcacgccgcaagacctgaaatcgttctgacccagagtccagcgacgctgagtctgagtccgggtgaacgcgcgacgctgagttgccgtgccagcgaaagcgttagcgtgcctggcatatctttcatccactggtaccagcagaaaccgggccaagccccacgtctgctgatctatctgggacgcaatcgggcggccggcattccagcccgctttagcggcagcggtagcggtaccgattttacgctgaccatcagcagtctggagccagaagatgccgccatctactactgtttacagagcagaaggtttcctcgacacttcggccaaggtaccaaactggaaatcaagggatccaccagcggctccggaaagcccggttccggagagggcagcacaaagggccaagttcagctcgtgcagagcggcgccgaggtgaagaagcccggcgcttccgtgaaggtgagctgcaaggccagcggatacaccttcgccgattacaccatcaactgggttcgtcaagctaccggtcaaggtctggagtggatgggctggatcaacaccgaaaccagagagcccacctatgcctacgacttcagaagtcgtttcacgttcactttaaacacaagcatcagcaccgcctatttagagctcagctctttaaggtccgaggataccgccgtgtactactgcgctcgtgacatcagatacgtgatggactactggggccaaggtacactggtgaccgtgtccagcaccacgacgccagcgccgcgaccaccaacaccggcgcccaccatcgcgtcgcagcccctgtccctgcgcccagaggcgtgccggccagcggcggggggcgcagtgcacacgagggggctggacttcgcctgtgatatctacatctgggcgcccttggccgggacttgtggggtccttctcctgtcactggttatcaccctttactgcaaacggggcagaaagaaactcctgtatatattcaaacaaccatttatgagaccagtacaaactactcaagaggaagatggctgtagctgccgatttccagaagaagaagaaggaggatgtgaactgagagtgaagttcagcaggagcgcagacgcccccgcgtaccagcagggccagaaccagctctataacgagctcaatctaggacgaagagaggagtacgatgttttggacaagagacgtggccgggaccctgagatggggggaaagccgagaaggaagaaccctcaggaaggcctgtacaatgaactgcagaaagataagatggcggaggcctacagtgagattgggatgaaaggcgagcgccggaggggcaaggggcacgatggcctttaccagggtctcagtacagccaccaaggacacctacgacgcccttcacatgcaggccctgccccctcgctaa

SEQ ID NO: 101 - DNA, 1473 bp, Artificial Sequence
  hBCMA-22 CAR
atggctctgcctgtgaccgctctgctgctgcctctggctctgctgctgcacgccgcaagacctgaaatcgttctgacccagagtccagcgacgctgagtctgagtccgggtgaacgcgcgacgctgagttgccgtgccagcgaaagcgttagcgtgcctggcatatctttcatccactggtaccagcagaaaccgggccaagccccacgtctgctgatctatctgggcagcaatcgaccatccggcattccagcccgctttagcggcagcggtagcggtaccgattttacgctgaccatcagcagtctggagccagaagatgccgccatctactactgtttacagagcagaaggtttcctcgacacttcggccaaggcaccaaactggaaatcaagggatccaccagcggctccggaaagcccggttccggagagggcagcacaaagggccaagttcagctcgtgcagagcggcgccgaggtgaagaagcccggcgcttccgtgaaggtgagctgcaaggccagcggatacaccttcgccgattacaccatcaactgggttcgtcaagctaccggtcaaggtctggagtggatgggctggatcaacaccgaaaccagagagcccgcctatgcctacgacttcagaggtcgtttcacgttcactttaaacacaagcatcagcaccgcctatttagagctcagctctttaaggtccgaggataccgccgtgtactactgcgctcgtgacatcagatacgtgatggactactggggccaaggtacactggtgaccgtgtccagcaccacgacgccagcgccgcgaccaccaacaccggcgcccaccatcgcgtcgcagcccctgtccctgcgcccagaggcgtgccggccagcggcggggggcgcagtgcacacgagggggctggacttcgcctgtgatatctacatctgggcgcccttggccgggacttgtggggtccttctcctgtcactggttatcaccctttactgcaaacggggcagaaagaaactcctgtatatattcaaacaaccatttatgagaccagtacaaactactcaagaggaagatggctgtagctgccgatttccagaagaagaagaaggaggatgtgaactgagagtgaagttcagcaggagcgcagacgcccccgcgtaccagcagggccagaaccagctctataacgagctcaatctaggacgaagagaggagtacgatgttttggacaagagacgtggccgggaccctgagatggggggaaagccgagaaggaagaaccctcaggaaggcctgtacaatgaactgcagaaagataagatggcggaggcctacagtgagattgggatgaaaggcgagcgccggaggggcaaggggcacgatggcctttaccagggtctcagtacagccaccaaggacacctacgacgcccttcacatgcaggccctgccccctcgctaa

SEQ ID NO: 102 - DNA, 1473 bp, Artificial Sequence
  hBCMA-23 CAR
atggctctgcctgtgaccgctctgctgctgcctctggctctgctgctgcacgccgcaagacctgaaatcgttctgacccagagtccagcgacgctgagtctgagtccgggtgaacgcgcgacgctgagttgccgtgccagcgaaagcgttagcgtgcctggcatatctttcatccactggtaccagcagaaaccgggccaagccccacgtctgctgatctatctgggcagcaatcgaccatccggcattccagcccgctttagcggcagcggtagcggtaccgattttacgctgaccatcagcagtctggagccagaagatgccgccatctactactgtttacagagcagaaggtttcctcgacacttcggccaaggcaccaaactggaaatcaagggatccaccagcggctccggaaagcccggttccggagagggcagcacaaagggccaagttcagctcgtgcagagcggcgccgaggtgaagaagcccggcgcttccgtgaaggtgagctgcaaggccagcggatacaccttcgccgattacaccatcaactgggttcgtcaagctaccggtcaaggtctggagtggatgggctggatcaacaccgaaaccagagagcccacctatgcctacgacttcagaagtcgtttcacgttcactttaaacacaagcatcagcaccgcctatttagagctcagctctttaaggtccgaggataccgccgtgtactactgcgctcgtgacatcagatacgtgatggactactggggccaaggtacactggtgaccgtgtccagcaccacgacgccagcgccgcgaccaccaacaccggcgcccaccatcgcgtcgcagcccctgtccctgcgcccagaggcgtgccggccagcggcggggggcgcagtgcacacgagggggctggacttcgcctgtgatatctacatctgggcgcccttggccgggacttgtggggtccttctcctgtcactggttatcaccctttactgcaaacggggcagaaagaaactcctgtatatattcaaacaaccatttatgagaccagtacaaactactcaagaggaagatggctgtagctgccgatttccagaagaagaagaaggaggatgtgaactgagagtgaagttcagcaggagcgcagacgcccccgcgtaccagcagggccagaaccagctctataacgagctcaatctaggacgaagagaggagtacgatgttttggacaagagacgtggccgggaccctgagatggggggaaagccgagaaggaagaaccctcaggaaggcctgtacaatgaactgcagaaagataagatggcggaggcctacagtgagattgggatgaaaggcgagcgccggaggggcaaggggcacgatggcctttaccagggtctcagtacagccaccaaggacacctacgacgcccttcacatgcaggccctgccccctcgctaa

SEQ ID NO: 103 - DNA, 1473 bp, Artificial Sequence
  hBCMA-10 CAR
atggctctgcctgtgaccgctctgctgctgcctctggctctgctgctgcacgccgcaagacctgacatcgtgctgacccagagccccgcttctttagctgtgtctttaggagagagggccaccatcaattgtcgtgcctccgagtccgtgtccgtgattggcgcccatttaatccactggtaccagcagaaacccggccagccccccaagctgctgatctatttagccagcaatctggagaccggcgtgcccgccagatttagcggaagcggctccggcaccgattttactttaaccatttcctctttacaagctgaggacgccgccatctactactgtttacagagcagaatctttcctcgtaccttcggccaaggtaccaagctggaaatcaagggatccaccagcggctccggaaagcccggttccggagagggcagcacaaagggccaagttcagctcgtgcagagcggctccgagctgaagaagcccggcgcttccgtgaaggtgagctgcaaggccagcggatacaccttcaccgactactccatcaactgggttcgtcaagctcccggtcaaggtctggagtggatgggctggatcaacaccgaaaccagagagcccgcctatgcctacgacttcagaggtcgtttcgtgttctctttagacacaagcgtgagcaccgcctatttacagatcagctctttaaaggccgaggataccgccgtgtactactgcgctcgtgactacagctacgccatggactactggggccaaggtacactggtgaccgtgtccagcaccacgacgccagcgccgcgaccaccaacaccggcgcccaccatcgcgtcgcagcccctgtccctgcgcccagaggcgtgccggccagcggcggggggcgcagtgcacacgagggggctggacttcgcctgtgatatctacatctgggcgcccttggccgggacttgtggggtccttctcctgtcactggttatcaccctttactgcaaacggggcagaaagaaactcctgtatatattcaaacaaccatttatgagaccagtacaaactactcaagaggaagatggctgtagctgccgatttccagaagaagaagaaggaggatgtgaactgagagtgaagttcagcaggagcgcagacgcccccgcgtaccagcagggccagaaccagctctataacgagctcaatctaggacgaagagaggagtacgatgttttggacaagagacgtggccgggaccctgagatggggggaaagccgagaaggaagaaccctcaggaaggcctgtacaatgaactgcagaaagataagatggcggaggcctacagtgagattgggatgaaaggcgagcgccggaggggcaaggggcacgatggcctttaccagggtctcagtacagccaccaaggacacctacgacgcccttcacatgcaggccctgccccctcgctaa

SEQ ID NO: 104 - DNA, 3294 bp, Artificial Sequence
  huBCMA-10-L6-Li CAR
atggctctgcctgtgaccgctctgctgctgcctctggctctgctgctgcacgccgcaagacctgacatcgtgctgacccagagccccgcttctttagctgtgtctttaggagagagggccaccatcaattgtcgtgcctccgagtccgtgtccgtgattggcgcccatttaatccactggtaccagcagaaacccggccagccccccaagctgctgatctatttagccagcaatctggagaccggcgtgcccgccagatttagcggaagcggctccggcaccgattttactttaaccatttcctctttacaagctgaggacgccgccatctactactgtttacagagcagaatctttcctcgtaccttcggccaaggtaccaagctggaaatcaagggatccaccagcggctccggaaagcccggttccggagagggcagcacaaagggccaagttcagctcgtgcagagcggctccgagctgaagaagcccggcgcttccgtgaaggtgagctgcaaggccagcggatacaccttcaccgactactccatcaactgggttcgtcaagctcccggtcaaggtctggagtggatgggctggatcaacaccgaaaccagagagcccgcctatgcctacgacttcagaggtcgtttcgtgttctctttagacacaagcgtgagcaccgcctatttacagatcagctctttaaaggccgaggataccgccgtgtactactgcgctcgtgactacagctacgccatggactactggggccaaggtacactggtgaccgtgtccagcaccacgacgccagcgccgcgaccaccaacaccggcgcccaccatcgcgtcgcagcccctgtccctgcgcccagaggcgtgccggccagcggcggggggcgcagtgcacacgagggggctggacttcgcctgtgatatctacatctgggcgcccttggccgggacttgtggggtccttctcctgtcactggttatcaccctttactgcaaacggggcagaaagaaactcctgtatatattcaaacaaccatttatgagaccagtacaaactactcaagaggaagatggctgtagctgccgatttccagaagaagaagaaggaggatgtgaactgagagtgaagttcagcaggagcgcagacgcccccgcgtaccagcagggccagaaccagctctataacgagctcaatctaggacgaagagaggagtacgatgttttggacaagagacgtggccgggaccctgagatggggggaaagccgagaaggaagaaccctcaggaaggcctgtacaatgaactgcagaaagataagatggcggaggcctacagtgagattgggatgaaaggcgagcgccggaggggcaaggggcacgatggcctttaccagggtctcagtacagccaccaaggacacctacgacgcccttcacatgcaggccctgccccctcgcgagggcagaggaagtcttctaacatgcggtgacgtggaggagaatcccggccctatgggggccgtcctgaggagcctcctggcctgcagcttctgtgtgctcctgagagcggagcagaaactcatctctgaagaggatctggaacctccaacatgttctcctcagcagtttacttgtttcacgggggaaattgactgtatccctgtggcttggcggtgcgatgggtttactgaatgtgaagaccacagtgatgaactcaattgtcctgtatgctcagagtcccagttccagtgtgccagtgggcagtgtattgatggtgccctccgatgcaatggagatgcaaactgccaggacaaatcagatgagaagaactgtgaagtgctttgtttaattgatcagttccgctgtgccaatggtcagtgcattggaaagcacaagaagtgtgatcataatgtggattgcagtgacaagtcagatgaactggattgttatccgactgaagaaccagcaccacaggccaccaatacagttggttctgttattggcgtaattgtcaccatttttgtgtctggaactgtatactttatctgccagaggatgttgtgtccacgtatgaagggagatggggaaactatgactaatgactatgtagttcatggaccagcttctgtgcctcttggttatgtgccacacccaagttctttgtcaggatctcttccaggaatgtctcgaggtaaatcaatgatcagctccctcagtatcatggggggaagcagtggacccccctatgaccgagcccatgttacaggagcatcatcaagtagttcttcaagcaccaaaggcacttacttccctgcaattttgaaccctccaccatccccagccacagagcgatcacattacactatggaatttggatattcttcaaacagtccttccactcataggtcatacagctacaggccatatagctaccggcactttgcaccccccaccacaccctgcagcacagatgtttgtgacagtgactatgctcctagtcggagaatgacctcagtggcaacagccaagggctataccagtgacttgaactatgattcagaacctgtgcccccacctcccacaccccgaagccaatacttgtcagcagaggagaactatgaaagctgcccaccttctccatacacagagaggagctattctcatcacctctacccaccgccaccctctccctgtacagactcctccgccaccaattttagcctgctgaaacaggccggagacgtggaggaaaaccccggccccatgcattggggaaccctgtgcggattcttgtggctttggccctatcttttctatgtccaagctgtgcccatccaaaaagtccaagatgacaccaaaaccctcatcaagacaattgtcaccaggatcaatgacatttcacacacgcagtcagtctcctccaaacagaaagtcaccggtttggacttcattcctgggctccaccccatcctgaccttatccaagatggaccagacactggcagtctaccaacagatcctcaccagtatgccttccagaaacgtgatccaaatatccaacgacctggagaacctccgggatcttcttcacgtgctggccttctctaagagctgccacttgccctgggccagtggcctggagaccttggacagcctggggggtgtcctggaagcttcaggctactccacagaggtggtggccctgagcaggctgcaggggtctctgcaggacatgctgtggcagctggacctcagccctgggtgccaccatcaccaccatcac

SEQ ID NO: 105 - DNA, 3294 bp, Artificial Sequence
  hBCMA-22-L6-Li CAR
atggctctgcctgtgaccgctctgctgctgcctctggctctgctgctgcacgccgcaagacctgaaatcgttctgacccagagtccagcgacgctgagtctgagtccgggtgaacgcgcgacgctgagttgccgtgccagcgaaagcgttagcgtgcctggcatatctttcatccactggtaccagcagaaaccgggccaagccccacgtctgctgatctatctgggcagcaatcgaccatccggcattccagcccgctttagcggcagcggtagcggtaccgattttacgctgaccatcagcagtctggagccagaagatgccgccatctactactgtttacagagcagaaggtttcctcgacacttcggccaaggcaccaaactggaaatcaagggatccaccagcggctccggaaagcccggttccggagagggcagcacaaagggccaagttcagctcgtgcagagcggcgccgaggtgaagaagcccggcgcttccgtgaaggtgagctgcaaggccagcggatacaccttcgccgattacaccatcaactgggttcgtcaagctaccggtcaaggtctggagtggatgggctggatcaacaccgaaaccagagagcccgcctatgcctacgacttcagaggtcgtttcacgttcactttaaacacaagcatcagcaccgcctatttagagctcagctctttaaggtccgaggataccgccgtgtactactgcgctcgtgacatcagatacgtgatggactactggggccaaggtacactggtgaccgtgtccagcaccacgacgccagcgccgcgaccaccaacaccggcgcccaccatcgcgtcgcagcccctgtccctgcgcccagaggcgtgccggccagcggcggggggcgcagtgcacacgagggggctggacttcgcctgtgatatctacatctgggcgcccttggccgggacttgtggggtccttctcctgtcactggttatcaccctttactgcaaacggggcagaaagaaactcctgtatatattcaaacaaccatttatgagaccagtacaaactactcaagaggaagatggctgtagctgccgatttccagaagaagaagaaggaggatgtgaactgagagtgaagttcagcaggagcgcagacgcccccgcgtaccagcagggccagaaccagctctataacgagctcaatctaggacgaagagaggagtacgatgttttggacaagagacgtggccgggaccctgagatggggggaaagccgagaaggaagaaccctcaggaaggcctgtacaatgaactgcagaaagataagatggcggaggcctacagtgagattgggatgaaaggcgagcgccggaggggcaaggggcacgatggcctttaccagggtctcagtacagccaccaaggacacctacgacgcccttcacatgcaggccctgccccctcgcgagggcagaggaagtcttctaacatgcggtgacgtggaggagaatcccggccctatgggggccgtcctgaggagcctcctggcctgcagcttctgtgtgctcctgagagcggagcagaaactcatctctgaagaggatctggaacctccaacatgttctcctcagcagtttacttgtttcacgggggaaattgactgtatccctgtggcttggcggtgcgatgggtttactgaatgtgaagaccacagtgatgaactcaattgtcctgtatgctcagagtcccagttccagtgtgccagtgggcagtgtattgatggtgccctccgatgcaatggagatgcaaactgccaggacaaatcagatgagaagaactgtgaagtgctttgtttaattgatcagttccgctgtgccaatggtcagtgcattggaaagcacaagaagtgtgatcataatgtggattgcagtgacaagtcagatgaactggattgttatccgactgaagaaccagcaccacaggccaccaatacagttggttctgttattggcgtaattgtcaccatttttgtgtctggaactgtatactttatctgccagaggatgttgtgtccacgtatgaagggagatggggaaactatgactaatgactatgtagttcatggaccagcttctgtgcctcttggttatgtgccacacccaagttctttgtcaggatctcttccaggaatgtctcgaggtaaatcaatgatcagctccctcagtatcatggggggaagcagtggacccccctatgaccgagcccatgttacaggagcatcatcaagtagttcttcaagcaccaaaggcacttacttccctgcaattttgaaccctccaccatccccagccacagagcgatcacattacactatggaatttggatattcttcaaacagtccttccactcataggtcatacagctacaggccatatagctaccggcactttgcaccccccaccacaccctgcagcacagatgtttgtgacagtgactatgctcctagtcggagaatgacctcagtggcaacagccaagggctataccagtgacttgaactatgattcagaacctgtgcccccacctcccacaccccgaagccaatacttgtcagcagaggagaactatgaaagctgcccaccttctccatacacagagaggagctattctcatcacctctacccaccgccaccctctccctgtacagactcctccgccaccaattttagcctgctgaaacaggccggagacgtggaggaaaaccccggccccatgcattggggaaccctgtgcggattcttgtggctttggccctatcttttctatgtccaagctgtgcccatccaaaaagtccaagatgacaccaaaaccctcatcaagacaattgtcaccaggatcaatgacatttcacacacgcagtcagtctcctccaaacagaaagtcaccggtttggacttcattcctgggctccaccccatcctgaccttatccaagatggaccagacactggcagtctaccaacagatcctcaccagtatgccttccagaaacgtgatccaaatatccaacgacctggagaacctccgggatcttcttcacgtgctggccttctctaagagctgccacttgccctgggccagtggcctggagaccttggacagcctggggggtgtcctggaagcttcaggctactccacagaggtggtggccctgagcaggctgcaggggtctctgcaggacatgctgtggcagctggacctcagccctgggtgccaccatcaccaccatcac

SEQ ID NO: 106 - DNA, 1824 bp, Artificial Sequence
  L6-Li nucleotide sequence
gagggcagaggaagtcttctaacatgcggtgacgtggaggagaatcccggccctatgggggccgtcctgaggagcctcctggcctgcagcttctgtgtgctcctgagagcggagcagaaactcatctctgaagaggatctggaacctccaacatgttctcctcagcagtttacttgtttcacgggggaaattgactgtatccctgtggcttggcggtgcgatgggtttactgaatgtgaagaccacagtgatgaactcaattgtcctgtatgctcagagtcccagttccagtgtgccagtgggcagtgtattgatggtgccctccgatgcaatggagatgcaaactgccaggacaaatcagatgagaagaactgtgaagtgctttgtttaattgatcagttccgctgtgccaatggtcagtgcattggaaagcacaagaagtgtgatcataatgtggattgcagtgacaagtcagatgaactggattgttatccgactgaagaaccagcaccacaggccaccaatacagttggttctgttattggcgtaattgtcaccatttttgtgtctggaactgtatactttatctgccagaggatgttgtgtccacgtatgaagggagatggggaaactatgactaatgactatgtagttcatggaccagcttctgtgcctcttggttatgtgccacacccaagttctttgtcaggatctcttccaggaatgtctcgaggtaaatcaatgatcagctccctcagtatcatggggggaagcagtggacccccctatgaccgagcccatgttacaggagcatcatcaagtagttcttcaagcaccaaaggcacttacttccctgcaattttgaaccctccaccatccccagccacagagcgatcacattacactatggaatttggatattcttcaaacagtccttccactcataggtcatacagctacaggccatatagctaccggcactttgcaccccccaccacaccctgcagcacagatgtttgtgacagtgactatgctcctagtcggagaatgacctcagtggcaacagccaagggctataccagtgacttgaactatgattcagaacctgtgcccccacctcccacaccccgaagccaatacttgtcagcagaggagaactatgaaagctgcccaccttctccatacacagagaggagctattctcatcacctctacccaccgccaccctctccctgtacagactcctccgccaccaattttagcctgctgaaacaggccggagacgtggaggaaaaccccggccccatgcattggggaaccctgtgcggattcttgtggctttggccctatcttttctatgtccaagctgtgcccatccaaaaagtccaagatgacaccaaaaccctcatcaagacaattgtcaccaggatcaatgacatttcacacacgcagtcagtctcctccaaacagaaagtcaccggtttggacttcattcctgggctccaccccatcctgaccttatccaagatggaccagacactggcagtctaccaacagatcctcaccagtatgccttccagaaacgtgatccaaatatccaacgacctggagaacctccgggatcttcttcacgtgctggccttctctaagagctgccacttgccctgggccagtggcctggagaccttggacagcctggggggtgtcctggaagcttcaggctactccacagaggtggtggccctgagcaggctgcaggggtctctgcaggacatgctgtggcagctggacctcagccctgggtgccaccatcaccaccatcac

SEQ ID NO: 107 - protein, 608 aa, Artificial Sequence
  L6-Li amino acid sequence
EGRGSLLTCGDVEENPGPMGAVLRSLLACSFCVLLRAEQKLISEEDLEPPTCSPQQFTCFTGEIDCIPVAWRCDGFTECEDHSDELNCPVCSESQFQCASGQCIDGALRCNGDANCQDKSDEKNCEVLCLIDQFRCANGQCIGKHKKCDHNVDCSDKSDELDCYPTEEPAPQATNTVGSVIGVIVTIFVSGTVYFICQRMLCPRMKGDGETMTNDYVVHGPASVPLGYVPHPSSLSGSLPGMSRGKSMISSLSIMGGSSGPPYDRAHVTGASSSSSSSTKGTYFPAILNPPPSPATERSHYTMEFGYSSNSPSTHRSYSYRPYSYRHFAPPTTPCSTDVCDSDYAPSRRMTSVATAKGYTSDLNYDSEPVPPPPTPRSQYLSAEENYESCPPSPYTERSYSHHLYPPPPSPCTDSSATNFSLLKQAGDVEENPGPMHWGTLCGFLWLWPYLFYVQAVPIQKVQDDTKTLIKTIVTRINDISHTQSVSSKQKVTGLDFIPGLHPILTLSKMDQTLAVYQQILTSMPSRNVIQISNDLENLRDLLHVLAFSKSCHLPWASGLETLDSLGGVLEASGYSTEVVALSRLQGSLQDMLWQLDLSPGCHHHHHH